European Patent Application EP 4 279 600 A1, published November 22, 2023. Title: Improved reactivity of nitrile hydratase with aldehyde. Applicant: Mitsubishi Chemical Corporation. The sequence listing filed with the application follows.

SEQUENCE LISTING (12 sequences)

SEQ ID NO: 1 - DNA, 32 bp, Artificial Sequence
  primer M8-1
ggtctagaatggatggtatccacgacacaggc

SEQ ID NO: 2 - DNA, 34 bp, Artificial Sequence
  primer M8-2
cccctgcaggtcagtcgatgatggccatcgattc

SEQ ID NO: 3 - DNA, 32 bp, Artificial Sequence
  primer PSN-1
ggtctagaatgaacggcgtgtacgacgtcggc

SEQ ID NO: 4 - DNA, 34 bp, Artificial Sequence
  primer PSN-2
cccctgcaggtcaggaccgcacggccgggtggac

SEQ ID NO: 5 - DNA, 1626 bp, Rhodococcus rhodochrous M8
atggatggtatccacgacacaggcggcatgaccggatacggaccggtcccctatcagaaggacgagcccttcttccactacgagtgggagggtcggaccctgtcgattctgacctggatgcatctcaagggcatgtcgtggtgggacaagtcgcggttcttccgggagtcgatggggaacgaaaactacgtcaacgagattcgcaactcgtactacacccactggctgagtgcggcagaacgtatcctcgtcgccgacaagatcatcaccgaagaagagcgaaagcaccgtgtgcaggagatcctcgagggtcggtacacggacaggaacccgtcgcggaagttcgatccggccgagatcgagaaggcgatcgaacggcttcacgagccccactccctagcacttccaggagcggagccgagtttctccctcggtgacaaggtcaaagtgaagaatatgaacccgctgggacacacacggtgcccgaaatatgtgcggaacaagatcggggaaatcgtcacctcccacggctgccagatctatcccgagagcagctccgccggcctcggcgacgatccccgcccgctctacacggtcgcgttttccgcccaggaactgtggggcgacgacggaaacgggaaagacgtagtgtgcgtcgatctctgggaaccgtacctgatctctgcgtgaaaggaatacgatagtgagcgagcacgtcaataagtacacggagtacgaggcacgtaccaaggcaatcgaaactttgctgtacgagcgagggctcatcacgcccgccgcggtcgaccgagtcgtttcgtactacgagaacgagatcggcccgatgggcggtgccaaggtcgtggcgaagtcctgggtggaccctgagtaccgcaagtggctcgaagaggacgcgacggccgcgatggcgtcattgggctatgccggtgagcaggcacaccaaatttcggcggtcttcaacgactcccaaacgcatcacgtggtggtgtgcactctgtgttcgtgctatccgtggccggtgcttggtctcccgcccgcctggtacaagagcatggagtaccggtcccgagtggtagcggaccctcgtggagtgctcaagcgcgatttcggtttcgacatccccgatgaggtggaggtcagggtttgggacagcagctccgaaatccgctacatcgtcatcccggaacggccggccggcaccgacggttggtccgaggacgagctggcgaagctggtgagtcgggactcgatgatcggtgtcagtaatgcgctcacaccccaggaagtgatcgtatgagtgaagacacactcactgatcggctcccggcgactgggaccgccgcaccgccccgcgacaatggcgagcttgtattcaccgagccttgggaagcaacggcattcggggtcgccatcgcgctttcggatcagaagtcgtacgaatgggagttcttccgacagcgtctcattcactccatcgctgaggccaacggttgcgaggcatactacgagagctggacaaaggcgctcgaggccagcgtggtcgactcggggctgatcagcgaagatgagatccgcgagcgcatggaatcgatggccatcatcgactga

SEQ ID NO: 6 - protein, 229 aa, Rhodococcus rhodochrous M8
MDGIHDTGGMTGYGPVPYQKDEPFFHYEWEGRTLSILTWMHLKGMSWWDKSRFFRESMGNENYVNEIRNSYYTHWLSAAERILVADKIITEEERKHRVQEILEGRYTDRNPSRKFDPAEIEKAIERLHEPHSLALPGAEPSFSLGDKVKVKNMNPLGHTRCPKYVRNKIGEIVTSHGCQIYPESSSAGLGDDPRPLYTVAFSAQELWGDDGNGKDVVCVDLWEPYLISA

SEQ ID NO: 7 - protein, 203 aa, Rhodococcus rhodochrous M8
MSEHVNKYTEYEARTKAIETLLYERGLITPAAVDRVVSYYENEIGPMGGAKVVAKSWVDPEYRKWLEEDATAAMASLGYAGEQAHQISAVFNDSQTHHVVVCTLCSCYPWPVLGLPPAWYKSMEYRSRVVADPRGVLKRDFGFDIPDEVEVRVWDSSSEIRYIVIPERPAGTDGWSEDELAKLVSRDSMIGVSNALTPQEVIV

SEQ ID NO: 8 - protein, 104 aa, Rhodococcus rhodochrous M8
MSEDTLTDRLPATGTAAPPRDNGELVFTEPWEATAFGVAIALSDQKSYEWEFFRQRLIHSIAEANGCEAYYESWTKALEASVVDSGLISEDEIRERMESMAIID

SEQ ID NO: 9 - DNA, 1747 bp, Pseudonocardia thermophila JCM3095
atgaacggcgtgtacgacgtcggcggcaccgatgggctgggcccgatcaaccggcccgcggacgaaccggtcttccgcgccgagtgggagaaggtcgcgttcgcgatgttcccggcgacgttccgggccggcttcatgggcctggacgagttccggttcggcatcgagcagatgaacccggccgagtacctcgagtcgccgtactactggcactggatccgcacctacatccaccacggcgtccgcaccggcaagatcgatctcgaggagctggagcgccgcacgcagtactaccgggagaaccccgacgccccgctgcccgagcacgagcagaagccggagttgatcgagttcgtcaaccaggccgtctacggcgggctgcccgcaagccgggaggtcgaccgaccgcccaagttcaaggagggcgacgtggtgcggttctccaccgcgagcccgaagggccacgcccggcgcgcgcggtacgtgcgcggcaagaccgggacggtggtcaagcaccacggcgcgtacatctacccggacaccgccggcaacggcctgggcgagtgccccgagcacctctacaccgtccgcttcacggcccaggagctgtgggggccggaaggggacccgaactccagcgtctactacgactgctgggagccctacatcgagctcgtcgacacgaaggcggccgcggcatgaccgagaacatcctgcgcaagtcggacgaggagatccagaaggagatcacggcgcgggtcaaggccctggagtcgatgctcatcgaacagggcatcctcaccacgtcgatgatcgaccggatggccgagatctacgagaacgaggtcggcccgcacctcggcgcgaaggtcgtcgtgaaggcctggaccgacccggagttcaagaagcgtctgctcgccgacggcaccgaggcctgcaaggagctcggcatcggcggcctgcagggcgaggacatgatgtgggtggagaacaccgacgaggtccaccacgtcgtcgtgtgcacgctctgctcctgctacccgtggccggtgctggggctgccgccgaactggttcaaggagccgcagtaccgctcccgcgtggtgcgtgagccccggcagctgctcaaggaggagttcggcttcgaggtcccgccgagcaaggagatcaaggtctgggactccagctccgagatgcgcttcgtcgtcctcccgcagcgccccgcgggcaccgacgggtggagcgaggaggagctcgccaccctcgtcacccgcgagtcgatgatcggcgtcgaaccggcgaaggcggtcgcgtgagcgccgaggcgaaggtccgcctgaagcactgccccacggccgaggaccgggcggcggccgacgcgctgctcgcgcagctgcccggcggcgaccgcgcgctcgaccgcggcttcgacgagccgtggcagctgcgggcgttcgcgctggcggtcgcggcgtgcagggcgggccggttcgagtggaagcagctgcagcaggcgctgatctcctcgatcggggagtgggagcgcacccacgatctcgacgatccgagctggtcctactacgagcacttcgtcgccgcgctggaatccgtgctcggcgaggaagggatcgtcgagccggaggcgctggacgagcgcaccgcggaggtcttggccaacccgccgaacaaggatcaccatggaccgcatctggagcccgtcgcggtccacccggccgtgcggtcctga

SEQ ID NO: 10 - protein, 233 aa, Pseudonocardia thermophila JCM3095
MNGVYDVGGTDGLGPINRPADEPVFRAEWEKVAFAMFPATFRAGFMGLDEFRFGIEQMNPAEYLESPYYWHWIRTYIHHGVRTGKIDLEELERRTQYYRENPDAPLPEHEQKPELIEFVNQAVYGGLPASREVDRPPKFKEGDVVRFSTASPKGHARRARYVRGKTGTVVKHHGAYIYPDTAGNGLGECPEHLYTVRFTAQELWGPEGDPNSSVYYDCWEPYIELVDTKAAAA

SEQ ID NO: 11 - protein, 204 aa, Pseudonocardia thermophila JCM3095
MTENILRKSDEEIQKEITARVKALESMLIEQGILTTSMIDRMAEIYENEVGPHLGAKVVVKAWTDPEFKKRLLADGTEACKELGIGGLQGEDMMWVENTDEVHHVVVCTLCSCYPWPVLGLPPNWFKEPQYRSRVVREPRQLLKEEFGFEVPPSKEIKVWDSSSEMRFVVLPQRPAGTDGWSEEELATLVTRESMIGVEPAKAV

SEQ ID NO: 12 - protein, 144 aa, Pseudonocardia thermophila JCM3095
MSAEAKVRLKHCPTAEDRAAADALLAQLPGGDRALDRGFDEPWQLRAFALAVAACRAGRFEWKQLQQALISSIGEWERTHDLDDPSWSYYEHFVAALESVLGEEGIVEPEALDERTAEVLANPPNKDHHGPHLEPVAVHPAVRS